European Patent Application EP 4 574 998 A1, published June 25, 2025. Title: METHYLATED BIOMARKERS FOR USE IN LUNG CANCER DIAGNOSIS. Applicant: Université de Franche-Comté. Application EP. The sequence listing filed with the application follows.

SEQUENCE LISTING (36 sequences)

SEQ ID NO: 1 - DNA, 5116 bp, Homo sapiens
  source 1..5116: mol_type = genomic DNA
  misc_feature 2501..2616: note = chr2:66438217-66438332
gagacgttaagggatttttcgtcgtgcttttttttttttttttttttttttccgggggagtttgaatatttgtttcttttcacactggccttaaagaggatatattagaagttgaagtaggaagggagccagagaggccgatggcgcaaagggtacgtattaaaaaacaattgtggaactcaaatgtgagattaaattgaaacgtggccgaaagacactgctaaaaagtttcctttttttctctctctcttttaaaaaatgaggctcctaaagccgtggcctaagcgagaggatttattcaatgcatttgtagacttatgtatgttacttggagttgttaattaaaggaatctatttatctatagattcctaaccagcagctatataaataaaaatgcaagctcaaacaatcatctgggtttttttttaaaaaagctagatacctaaagctgtaatttgaacattcagagatcagaagtttaaagttatgtttaaactaaaatatgcagctggaaacttctgatatgttattgattatgctcatctttaatatcactagaagtattcagctttttaaaggaaataactttgtcatagtatagccaattttttggtcagaaaacattcatctttttatagtaatttcaatttgtatagacttgtatacaaggcaatattttgcaagtttctcttagataagccctctactaattgaatactaagcacacagttactcactttaaaaatgcaatactaatttccccatattcctttttcaatggaaatgcagtgagagtaaagtgagacaatgacaacccaactgaggtagtttcttaaaagaaagggggtctacaaaaagccttccttgcataatttgtgtcctggccctcaaagccctgtttgcaaaagaaagttactaggctgacacagttttctttactcctttggttcaggcaaatgtcagcgttcttccaaactcttttcacacctctggctttaaggagatgaaagtggcaattcctcctttctttgaaaatcatttcactctcagcgcctccaaatcttgggaaaataactgcctggaatgaaccaattagaaaaacctaaatagctaaatttcacacacacaaaataatgacaatcaatatgaaagtagttttttttttttttttctggaagaggaagatggaaagttgtgcatttgcttttgaatttgctttaaacctggtgagtaacatttgcctccttgacttctagtctggaaacaaagttcataagagtaaataagaaaatagaatattagctgcttcaactatagattttctttaactttgggggtggggaattgcccaattctaaattcagctctgatgttcaggaaaagctaccctcctttgagtttcacttataaggggtcagttagttttgtataatttagcagagtttgtcttggaaagcaaaagaaatgcagtgtcttgtaggactgcctaacctcacgctggcagggaaataaaatgagaagcctgtctaaattcacgtgctttgcgtagctgttcccatcgtaacttttttttttttttttaattccccctgatgtgaaggggctgtgaaactaggcgggtttgctgcagtgtcctggcacgttttattattgtgattttgaatttcttcctccagagacatgcccgtttcaccttctaccctcgggagaatgcttctctttctctctttctttcttctttccttcttgccaaaggagcctgaatttctaaactagttgatagggacacaagttagggcaagatcattcatcccagacgagtctcgctgagaattctgtattttttacttaaagctttaattttaaaataagaaaaactcagctttatagatgcaaggccaccgaattccgggtggaaggacccagctgtattgaccttatataagctcggtgccttgccgttctcccatttgcccgcctggcctcctgaaccttctttctctcctgtttgtcatgcagtacgacgatctaccccattacgggggcatggatggagtaggcatcccctccacgatgtatggggacccgcatgcagccaggtccatgcagccggtccaccacctgaaccacgggcctcctctgcactcgcatcagtacccgcacacagctcataccaacgccatggcccccagcatgggctcctctgtcaatgacgctttaaagagagataaagatgccatttatgggtaggtacaatgggcagcaggttaagtagttgagactcaacgcttccctctttctctgtgcccttggtaagaggaaagtcagagttctctggattggaggtacatctttggtgacttttcattcacatttcatggataatttggggaggtggcctgccatccctgaagccctacatccccatacacactctgtgcacatccagtgccctgctccaccatggcagtgcccgcaagggggtcccagatgagaagaagctggctaaagggcccttgtcccctctcagactccttcagcgggctggagtcctccctcgctcgatttcgcccgagagcgttaggggtttctaaatgcaggcgcctttgtgttgtaacgaaacttttagtttaagggaaaatctcttttaagccactgattgttctgacttgctgagtttactcagcagccttatgctggctctgccactgcacaataaaaccaaagcaggacagttgcaggtcaagcaagggggaacatgttttgcatttagggagtttgaccactgaagtcaaggagaggagcttgctctgaattgttacacacattaagaaacttctagatgttttagcactttgtgctcaaaggcgaaacctgcaggatttagaaataagtaaattcggggtgctcttcctcggaggttgttttctggctgcggtttatactgctttctcctccgccattcgattagaccctgggctagtagaatcctttgaaactcacttgtgcctactgtgtgccgatgaatttgggaacctctttttactttgcagaaacttttatttctatttatttatttttaaaaaatcaggacacactgaccctccctcgctggaaaaaaaaatatatataatctttttattttattttctgatcccttgtgcgatgggcttgtttaattcccaccgttctgtccgcagagttaactacaagtggtttaggctctgggacagaacatttggggaagctttgtaaaggaccccaaactgttaaattcccagctgagctgtgagagctaataaaagacttgagatacctccttgggcattagaagaagcttttctttctttcttcttcttcttcttttttttttttttttcttttttatgggctgagacaagcgacatctaggcccctcgcaatactagctgctttgccacttcgcagagacaaaatgaaaggctctactgcaggaacatttgaaggaactttctttggggggcggtgggggctatcagcgaagggaggggaatgtgcgtggagctgaggaggagcctcccggctctccgagggccttggggttgggatccctaggtgcagcccgttgacagtcggccccacggccatggacgtcctttccccaagttagctgagcgcctgccaccgagatcccccgagcctgggcttcgcgcggccgcctaggaggaacccgcaggaaccagccctccccaactctccgcccggcgcctttctcctccaccggatcctggatgtgcagtggaggggacgagggcttgtcgggtgggaaacttaattcaaaatggctgctggaaacgcttgggttttattcgtagcaaatgttgccaatttctccggccagatacgctaaaccgatcctcagataccgtccatggctcagggcctccgacttcagggctccaggaggaaggggaggtgagcggtcacctgggtctgggggagggggaggaaaaggaaaaaagtagatgacacaatcggagagggggtctgttcctcttgctcctccagctgtttttcttgggcacctttttccattgactggggactaaccattatgttgtttgtgactgttgtattttcttgcagacaccccctcttccctctcttagcactgatttttgagaaatgtgaattagctacttgtaccccccgcgagccgggggtggcgggcggggacgtctgctcgtcagagtcattcaatgaagatatagccgtgttcgccaaacaggtcagcaaaatagatgttaaaaagtaaaagaaacaaaaagagagcccccccttcgccaacacacacgcgcgcgcgcgcgcgcgaacacacacacacacacacacacacggcacactttcaaaagtagccagcacgtagtcggccttaagccatgcatgttacctccaacctcagattttctctctgtctgagtgtctgtttgcagataacttaaaatcacccatctgcatccccactcaccctccagaaagcaaacgtggagagctcactctgcagaataaaatcaagaacaccacggttgtagctgctgtggactcggcggtctgagcagcctccccgagagccgtagttgctagtagaagtaagattgagctctgggcttgttttcagcttatttaattcacactgaaatgtttctgcgcgggacgaactcggtgtcaccgggtccctcccggagggttacttcctgcccccgacagtgtaatgaggcaagaaactaggaaggcgaccagatttcaaatttttctttcttttttctctcccctccctctcccctctccttctcacttgtatttagattcgcgcagaaaaacctctattttcttctaatccagaactggataacttggtaagagcggacccctatttccctcccccgcccccgaccccctacctcccacctccaacgccctcagctttgctttgagagccctgagatttctagaccggtcttcccgtgcctgcaggttggctgcaaatgtttctgtacacggacaactggtccgggacaagatcccggggaaataaattcatctcgagaggggccgggcgagccagcgcggggaaac

SEQ ID NO: 2 - DNA, 5077 bp, Homo sapiens
  source 1..5077: mol_type = genomic DNA
  misc_feature 2501..2577: note = chr8:96159758-96159834
gggagaagtggcctgggatggagtacagaacttgctttctttataaacctaaagcgtccttcattcactttgggcagagtttatgcctgttctcccactctcaaccataggcttcaggtgtaactttggggtttccggggtaaggaaggctttttacagatactgtacaggagcaagtcgcccatgcctcctggactgacttcggggctcctttccttttcttcgctcctccccttgggggacccccggctccaccgagccaggccagccccactcgacggcgatttaaacatcccttaggcaaggcgccaagttagcgctgctggcccagctctaggcgggccgctgctctttcctcctcgccaggccgtccacgcgttgggggaggggaccctaggggggttggcgcggttaagagccccacgtgagaggggcggaagtccttgccaggagccggggatgcgcggctggcgggtcccttccatcacgggagacgagacaccgtttgatgtgttatgacatgaaccctcaattagatcgctgagttgaaacactccaatcaggggcccgatgctaagcaagccccggaaggtccagcctgaggtcaccgccggtgacacatcaaatcaaaatcagtgagagggaaagtgaggctttccctttatcaagctggggctgcagccagcaacgcaccccctcctctgcgcacccctcccgcccgtggctccgcactccttcacccccgcgcggcgtgcgacaagccgcaccgccttcccagtcaacgaactgcctttcttcgcattttctgagaacccggagacgcggaggagacagcgcctttgaagatgctgtccgggtggtcatgcagcgtctcctcccgctgtggaccgctcgcatccccagccctccaccgcattccggggttgtagcggtacttgtggatctcggtcctgctagtctggaggccttggctcgggaacagaggcctccccagactgggtgcacatgcaatccctcctctatctccaggatcgggggcatacagcgcagtggcggggatgggggtggggaggctacagggcaaaccagggtaaagtgatttcgcgtctacgccggattggggcccccaagacttttccccaacccttgtctgaatgccacaggcttccggagacacctccgaacagcccgcagggtcttttggtcctgtgccaaattcacagggcgcagcgaaccagttatggtgcccacttgggggaggggcagagattcttgccacttcattcccgggcaaagaaaatccgcgcccaaccgccggccagcctaggcctctgggacttcttctcttgaggaagggcctcttgagcagtcttctctgagcttccttagcctccttccgcaattgtagtagagaaagtgcacgattaacagaggactttgagggacagaaacaactgtagcaaggcgtgcgtcgtggggagggttggcgagctgcacgggcagcacggaggccagggactcagttgcactactacgaagaagccacatgtctttgcaaaggtgactttagtagccctaaaatcatcataaaatacctggcgttaatttgccctctggacctttcagcagctcatgaacctcgctgacctcgggctgcagcggcgagaccctcgagcaaggaacgcgactatgagtgagaggcggggactggagccggggaagagctcggggctgggggcgggggggccgttagcctgctctaaaaagcttaagagatgtgcgagcacccagggtagcagtggctgaagcagcttccgaatcccgaaccccagcgctgcaaggtttccgggcaaccccacttaactgggagcaggtcaaagtcatggagctaagtctagggaggatggaggagtggatatctgcctaaatcgcttttatcccgtcattttcttccttccttctctttactcttcctttcctttttctcccttcctttcctgtctccttccacattattgtctctctcctttaggagcttagtttccgatgcctgtggatccttccctgatttctgggaccagaggtggtgcgaggttttcttgagggcactggccacgctgcagatcaacgccggtggcaagaaggggccgcaagggtttccgcagacacccacacatgcaggcgttcccacagagggtaccagggatttcccagacccccaccagccctcaggaatagcgtagagagaggaacgtcgcctggctgagaaaggtggatgggcatacccatgtacctttgtgtattaagtacccacaacctccgaacttagccgtccctgtcccggcccgcccaactgctgccgccgcatctgcagaaaccactcgtgttgaggcctcggagcagccgggagcaccacgctggagcaaaaaagccggagggcgcagggctccagcccggctgaccatcccacccagcgcagggaccaacggaaaacccgcgcggcgccaggaccagggggctgcccgacgccgctcgcggactagttcctcagactgtgggactccctagtgccggctttgcccagggctttccaaggctgtctcatgccctagatctgccccagcagctcaggccttggactgcgaacccagtatcccgagacaccgattccatcagtccccatcccgacccctctccagccgggttcatccgcctgctgcctcccgtcctccacgtttcccccaccagccaccaacaagcggcaaccacgctgccttctgcaaaagaggaagaaggaaagaagggagagagaaagaaagggggggaaaggaagggaggtttagagactggaatagaatccgcagccacattcagaaacttactcgagcttgagaaaaacaatttaagaaaagtaaaaaggaagtgtccagagcaggaagggaattcacaaatgtagcctccagcgggaacagctccctggctgccgagctccagcgggaggggagtcgagcgttttctttgccacttacctagtcccctgtctacaaagctggtgatcgtattagccgacttggaagactggaaaaagctggcattgatgcccagcttctcagcgatggagtaagtcctgtagattgacagcatgtactcgtggggcaccacgcgcggacccctgcctggcggctcctgcgcccggggctgctgagcccggggttcgtcctgaggccgcggctgtggttcctggccctcccggcccgcgtcactgtcgcgcggcgcccgctgcatcttgccttccttgcggcttcgcatgcccttggtggaacccagctcggcggacgacgaggaggatgagatggaagcctgctggaaaccgggcaaatcccacagaaaactgatgaggaagacggccgagagcaggaccctgggagtatccatggcgggcaagtggctgcgtctccccaggaggcggtggcggcggcgcaggacgcgcggggcacggagcggctggacagcggccggggcccggctcctcgggcggactcggagtgcgaggagccgggtcccagccacacaaaccccggccccgccacgccccctcccgcccctcgccgggaggggaggaatggggagggagggcagaggaggggtggggagggtgggaggagagccgggtggtgcgggccggaggtgtgggggagaggggccgcggtgcgccggtgtggcaggaagacgcagcgcccccgcgggacgcgcgcggggttgccgggcggtgcgcgcggcgcgggccgcaagcgctgaccgggggaaggcgggcgctgccggcccgtggccggggagcaaaggctggcccgccgcgccagggtccccctcgaactcccggaggtgtggtccctccgcagcgcggccccggctctcggtcctcgccagccgcctccactttcctgggagcgagcggccccggaggagggaagcggcggcggcgcccccaagagacagcttggagcaggcgcctctgctgcaggctgcgtgctgcctcggggcggtggtaccctccctcctcggccccaaccgccaggcctgccgtttgcgcccctcaggggccagcccggagccagagaagcctcgccctgggccaggcgcagggcccagctcggaacagccccattttctcggttgggtatcgctctccacaaagacaggcgtctattcccgaccctcgaggtcaggcaaaggccacgagtctttagagtttggatcgatgctaaaagctgctgcgctcccctgcaggccccagcctctcctctcgcagtccccaacctcttctgacgcagactttagctgctccacttcttcgtctgctcccgggatcctctccctctcgcggcctgccccccgcctccactgcatccccattttccctctcttctttccctcccgcctgcaggacttcctccttccccaagttccttctgcattccaatccctcttccccagcctgcttttcttctcacactgccctcccatctcacactgccttcccaccctctctcttcccggcctcccccctcgccttccagtggacccctccctttgcagctctaccccaatctgtttctcttcagcccagcctcgccccatcacgagtttcctttatctgtccccagattccccgtgcctgtcttccccgcccactgcctcgctcattcctgggcctgcacgctgaaaggcgatgcggcgtagcgctgcttctgtctgccacagtgctctgccctggactgctatgggcagaagagtttccctcagtactgattgggtgctcaggcaccaaccataaagtaccctcctttaatcgtgccaacagctttgtgaggttggcgttgactattttcaccttcacggatggaaaaaaaaaagactcaatggaaataagtgacttttccaaggccactctgccaagaggttatgcagcaagggacagaacccaggctcccaccccaagcccaagattcttcccactacagcatagacagtcattcctggcccaacttctctatttcagttctggcttttttcttct

SEQ ID NO: 3 - DNA, 5089 bp, Homo sapiens
  source 1..5089: mol_type = genomic DNA
  misc_feature 2501..2589: note = chr17:48633954-48634042
ctggccctccaagtcagcctggcgccgaagccccatccggtcgggcctctttcccgggcccctttgcacatttcctctgcctcaagcagcagggggaaggtttgggaacaaaagttagcttatgctttggaaagtcccccttcttccaccagcacttctagttattcctttcctgggcacagggccaacagccttaagaggaccgaggtcagagagggtatcagagtcttgccctgcccaacccctggtttcatcccttgtcactgcatcagtcggggttgaattgtccaacaacctgggctccccattagcttgcaagtcaggcccctctccaaggaggtggcactcaggacctatgtgtacccccagcccagcccaaggccagtgggaagcctttggccactggggtgggtggggaggaaaaagtcaactgagggattaggaaaggaaggacttttcggacctacttctgtaggtctggtcccatagggggccttcgacaggaccctgagggctttaggctgagattgcaagagctctcagtgtttgcctttcagaatgagacctactgagccctcttcaaggacctgaagcttcctgctgaggtggagcaccagcccgcaaagagttacaaaaacctcaagaaccccctgcatttcttttgaaatcaaatatttgtgaagttggggagagtttctctggaaagttctggatgtagttgagagctcagagaccctaaggctggaagttggagctctgactgccatctttgggttgggctgaacagcccaacagggccagggaggtgcctcgggagagttgactgctcctcatcccccttcccctcctaacacacacacaaaaaaacattcagaagtgggaagacacttcccagatctcttctctgggggaacatccttgttgctcctggatgaaggacctcaaacctcttccccattttgcaaggttgatcttccagtcctgattctgctcccctcccccaactcctccagctaagcaaggagcagtaactgccgtgaatcgggtggtttaatgttgttgtgttcagaaacccaggcccaacaacatgaaactacctaattcactcagcagttccaattcaagctctaggtcaagagctcactgggggcaaaccctgtggccatttttttgtgggccaaaaagcggcttaacttcattttgctccacctcttccccaacagaagaacccagttgctactaaacaacacatcggaagaactgaacccaggactctaggtaaaaccattttggagccggtcctgatagctcagattccagagacatttgctgccttccaggagccctggccagagaagaagaccctagacacaggcacaagcctgggcagggcctctttgatatacctgctcagtctctgcctctcagcccagctggaggtctccacagataaaaagaattctcaacttcaaacagatacgaaggtgcatctatactcagcaccctgctagcccctgtattccaggtcacccagcctcccagtgtagctctgagaggccagatcttcaagtcctacacaccccccagctttgagattggggctcagacaggagagtgagacaaaagagtgctgagaaagaaagtgacagagagaaaggtggaaaagcagagtgtcagaaagtttcgggaattctagggaacaaacagaggaagaatgggatttggaggggaaagccggttgatctgaacagttgctgtgaaggcaccctgcccaaaatgtcccagggccctggctctgcagaggccgagctgccccaggtaagacaattcattccgaatcttcgcagaataaggactgagaggctaaggactgggattgggacacagagaacaaatttgcttcctccttcctgaccttcggtctgggtccttggccccctaacgtgcccgctcctcacctctgcctctccagacacccgcctgctcacaggtgctcacgctcacacccgcacccatcgcaaaaacgcagctgtgcaggccgagggcggcggcggacttacctgggcggcggcggtgccggcagtgcgcggccgtcggaaggtgcggagccagcggccgcggcccagtccaggctccctcccgccctcgcccagaagcgagggtccgagtggccacgtgtccggcagggaagtccgaggtagcgagggagtccacctggccgcccgctccccctcccgggtataaatcttggggaccggaaatacaataaaacttcaccgtgttgatgaacttcaaacggtttacatcccctcctgtcctgaaaagaaagacgtccgggggcggattaaaaggaaggggaaacaaatttacgagcggcagaagcacccgcctcggcccctttctttgcccgcacactttgtccgcgtggagagaagcagccccagcccccgggacttggcctccgccgaaccggccgccaggcgcgctcttctctcggaggagtcggcgctgacccagcccgcgcccggcagagactggaagccgccgcctacacggaaaatccacagagccccgcgcagaccctatgatcggctcggcccgccgggcttgggatgaggctccctgcttctcgctagagcagaactgggctccctggcgcttccttgcgaaagcccaggctctcccaaccacgcccggtggcctccattttttgcatctttccgctgaaagcgggttttttcttttttctttttttttgacagagtcctgctgtgtcacccaggctggagtgcagtggcgcgatctcggctcactgcaacctccgcctcccggttcaagcgattctcctgcctcagcctcccgagtagctggaactacaggcgcccgccaccacgcccggctaatttttgtatttttagtagagacggggtttcacaatattggccaagctgatcttgaactcctgacctcgtgatccaccctcctcggcctcccaaagtgctgggattacaggcgtaagccaccgcgcccgacccaagggttttttgtttttgttttttgtttaactttacttttctctttccttttccgtttctagcggccagacctttgcccagccctgcccgtttattgccgggtacttgctggaaggggacagaagataagactcggggtgactcccaaggcctgaagggggctgattgggccgggggctcccagaggataaacctaggggccggtcggtcttcctcggcgtggaagtgagagccacgcggcgtggcggagctccaccaccgtctccttatctctttaaagcctcaaaatcaaacaaaaccactactacccaggcctcaagtttccacagtttttgtctgctctggaccgtttactttttttgaaaaaagagaacttggtggaatccaaattctctactaggcctccgaaccaaaacgaaggaaaatccgttttcttcttgggcttcagagaactgggatcgaagtgattgacttcctgctccttttgtctgctccaggggcctggttaggtgcccttctggatgggagagcaaaaggttctccatcctgcctcacagttattcacctccaaaacagttttgagacacaatggatggctaagattagctcaggctcaggcagagtgttcaggtacaggagtgaggtccagctgcaggcccaagagggggtttagtgcactgaaggcacccaccttcccatagatacacacatagataaccccactccccaaccccaagaaaaggcaccaaagtgctgctggatattttaaaaatctgattaaaaaataaacgggcagggaaaatactaggcagtataggttttgaattttctgaagggttaactctgctgcaggcagtcccactcggccccagctctccagaggtgggtggtggtctgggggcagtgccctctggccccttcctagcaccaaaagggaggaattggggagctctttaacagctggagggcaggaagtatcttatttctggccaacattcatattccagtatttgcatggggaggcccctccagcctccctcatttgctctttatcatgttatattttcattcaaaatactgagatggcagctactggctgtcacttcttctattaggatttccctctgggaggacggcaggactgaggggccagcagtttccagaccattcaagagtgttattacccatcccctaccgggcacctggtgggggccggtgtgctggctcccagcctactgctggcctgggtctctgtggctccctggctgagaaaaggagatggaaaccttttatagtcttagactctttggaaaaactgaagaggccatagccttaggatgatgcacctgcacacccatatgttttgcatacatttccaggggctttgtggcttccccctacccccatcccaagaacccaggccatggattccaattaaaaaaacaaaattatctgtatggtgccaaaggacaccccaaagccattcccatagataccagctgtgtctttccgagggctccccaaaggataagtcaactttcagaggctcagcacagacacccatggccggggtgctggtgccgctcatacactaactagctgagatgatggtcactccgtgagtaaaggccagttaggcaacatttcttttcacccccaaacgttttccaaacacttttccaaaagcatgttgacctccaaattattcagaaaattgatggccatgctggagggtttagaggtaacttctccccactccctttcttccttgaagataaagcagagttctagcgtaactggaggggggctagacaatttggttggtgagaggaggcagtgtagacacagacgcagaacacaagttccttaaagaaacaaaaattgagacccttttccattttgtgagagtcacaagaataaatatttctgggacttcctggcctgtctcccttcacagggttcattacaggcggggagggaggagacagtctcggagaattcagaggtgccagaagccgagttcctagaccccagctggattttttttttttttt

SEQ ID NO: 4 - DNA, 3116 bp, Homo sapiens
  source 1..3116: mol_type = genomic DNA
  misc_feature 1501..1616: note = chr2:66438217-66438332
ggagatgaaagtggcaattcctcctttctttgaaaatcatttcactctcagcgcctccaaatcttgggaaaataactgcctggaatgaaccaattagaaaaacctaaatagctaaatttcacacacacaaaataatgacaatcaatatgaaagtagttttttttttttttttctggaagaggaagatggaaagttgtgcatttgcttttgaatttgctttaaacctggtgagtaacatttgcctccttgacttctagtctggaaacaaagttcataagagtaaataagaaaatagaatattagctgcttcaactatagattttctttaactttgggggtggggaattgcccaattctaaattcagctctgatgttcaggaaaagctaccctcctttgagtttcacttataaggggtcagttagttttgtataatttagcagagtttgtcttggaaagcaaaagaaatgcagtgtcttgtaggactgcctaacctcacgctggcagggaaataaaatgagaagcctgtctaaattcacgtgctttgcgtagctgttcccatcgtaacttttttttttttttttaattccccctgatgtgaaggggctgtgaaactaggcgggtttgctgcagtgtcctggcacgttttattattgtgattttgaatttcttcctccagagacatgcccgtttcaccttctaccctcgggagaatgcttctctttctctctttctttcttctttccttcttgccaaaggagcctgaatttctaaactagttgatagggacacaagttagggcaagatcattcatcccagacgagtctcgctgagaattctgtattttttacttaaagctttaattttaaaataagaaaaactcagctttatagatgcaaggccaccgaattccgggtggaaggacccagctgtattgaccttatataagctcggtgccttgccgttctcccatttgcccgcctggcctcctgaaccttctttctctcctgtttgtcatgcagtacgacgatctaccccattacgggggcatggatggagtaggcatcccctccacgatgtatggggacccgcatgcagccaggtccatgcagccggtccaccacctgaaccacgggcctcctctgcactcgcatcagtacccgcacacagctcataccaacgccatggcccccagcatgggctcctctgtcaatgacgctttaaagagagataaagatgccatttatgggtaggtacaatgggcagcaggttaagtagttgagactcaacgcttccctctttctctgtgcccttggtaagaggaaagtcagagttctctggattggaggtacatctttggtgacttttcattcacatttcatggataatttggggaggtggcctgccatccctgaagccctacatccccatacacactctgtgcacatccagtgccctgctccaccatggcagtgcccgcaagggggtcccagatgagaagaagctggctaaagggcccttgtcccctctcagactccttcagcgggctggagtcctccctcgctcgatttcgcccgagagcgttaggggtttctaaatgcaggcgcctttgtgttgtaacgaaacttttagtttaagggaaaatctcttttaagccactgattgttctgacttgctgagtttactcagcagccttatgctggctctgccactgcacaataaaaccaaagcaggacagttgcaggtcaagcaagggggaacatgttttgcatttagggagtttgaccactgaagtcaaggagaggagcttgctctgaattgttacacacattaagaaacttctagatgttttagcactttgtgctcaaaggcgaaacctgcaggatttagaaataagtaaattcggggtgctcttcctcggaggttgttttctggctgcggtttatactgctttctcctccgccattcgattagaccctgggctagtagaatcctttgaaactcacttgtgcctactgtgtgccgatgaatttgggaacctctttttactttgcagaaacttttatttctatttatttatttttaaaaaatcaggacacactgaccctccctcgctggaaaaaaaaatatatataatctttttattttattttctgatcccttgtgcgatgggcttgtttaattcccaccgttctgtccgcagagttaactacaagtggtttaggctctgggacagaacatttggggaagctttgtaaaggaccccaaactgttaaattcccagctgagctgtgagagctaataaaagacttgagatacctccttgggcattagaagaagcttttctttctttcttcttcttcttcttttttttttttttttcttttttatgggctgagacaagcgacatctaggcccctcgcaatactagctgctttgccacttcgcagagacaaaatgaaaggctctactgcaggaacatttgaaggaactttctttggggggcggtgggggctatcagcgaagggaggggaatgtgcgtggagctgaggaggagcctcccggctctccgagggccttggggttgggatccctaggtgcagcccgttgacagtcggccccacggccatggacgtcctttccccaagttagctgagcgcctgccaccgagatcccccgagcctgggcttcgcgcggccgcctaggaggaacccgcaggaaccagccctccccaactctccgcccggcgcctttctcctccaccggatcctggatgtgcagtggaggggacgagggcttgtcgggtgggaaacttaattcaaaatggctgctggaaacgcttgggttttattcgtagcaaatgttgccaatttctccggccagatacgctaaaccgatcctcagataccgtccatggctcagggcctccgacttcagggctccaggaggaaggggaggtgagcggtcacctgggtctgggggagggggaggaaaaggaaaaaagtagatgacacaatcggagagggggtctgttcctcttgctcctccagctgtttttcttgggcacctttttccattgactggggactaaccattatgttgtttgtgactgttgtat

SEQ ID NO: 5 - DNA, 3077 bp, Homo sapiens
  source 1..3077: mol_type = genomic DNA
  misc_feature 1501..1577: note = chr8:96159758-96159834
tgcacatgcaatccctcctctatctccaggatcgggggcatacagcgcagtggcggggatgggggtggggaggctacagggcaaaccagggtaaagtgatttcgcgtctacgccggattggggcccccaagacttttccccaacccttgtctgaatgccacaggcttccggagacacctccgaacagcccgcagggtcttttggtcctgtgccaaattcacagggcgcagcgaaccagttatggtgcccacttgggggaggggcagagattcttgccacttcattcccgggcaaagaaaatccgcgcccaaccgccggccagcctaggcctctgggacttcttctcttgaggaagggcctcttgagcagtcttctctgagcttccttagcctccttccgcaattgtagtagagaaagtgcacgattaacagaggactttgagggacagaaacaactgtagcaaggcgtgcgtcgtggggagggttggcgagctgcacgggcagcacggaggccagggactcagttgcactactacgaagaagccacatgtctttgcaaaggtgactttagtagccctaaaatcatcataaaatacctggcgttaatttgccctctggacctttcagcagctcatgaacctcgctgacctcgggctgcagcggcgagaccctcgagcaaggaacgcgactatgagtgagaggcggggactggagccggggaagagctcggggctgggggcgggggggccgttagcctgctctaaaaagcttaagagatgtgcgagcacccagggtagcagtggctgaagcagcttccgaatcccgaaccccagcgctgcaaggtttccgggcaaccccacttaactgggagcaggtcaaagtcatggagctaagtctagggaggatggaggagtggatatctgcctaaatcgcttttatcccgtcattttcttccttccttctctttactcttcctttcctttttctcccttcctttcctgtctccttccacattattgtctctctcctttaggagcttagtttccgatgcctgtggatccttccctgatttctgggaccagaggtggtgcgaggttttcttgagggcactggccacgctgcagatcaacgccggtggcaagaaggggccgcaagggtttccgcagacacccacacatgcaggcgttcccacagagggtaccagggatttcccagacccccaccagccctcaggaatagcgtagagagaggaacgtcgcctggctgagaaaggtggatgggcatacccatgtacctttgtgtattaagtacccacaacctccgaacttagccgtccctgtcccggcccgcccaactgctgccgccgcatctgcagaaaccactcgtgttgaggcctcggagcagccgggagcaccacgctggagcaaaaaagccggagggcgcagggctccagcccggctgaccatcccacccagcgcagggaccaacggaaaacccgcgcggcgccaggaccagggggctgcccgacgccgctcgcggactagttcctcagactgtgggactccctagtgccggctttgcccagggctttccaaggctgtctcatgccctagatctgccccagcagctcaggccttggactgcgaacccagtatcccgagacaccgattccatcagtccccatcccgacccctctccagccgggttcatccgcctgctgcctcccgtcctccacgtttcccccaccagccaccaacaagcggcaaccacgctgccttctgcaaaagaggaagaaggaaagaagggagagagaaagaaagggggggaaaggaagggaggtttagagactggaatagaatccgcagccacattcagaaacttactcgagcttgagaaaaacaatttaagaaaagtaaaaaggaagtgtccagagcaggaagggaattcacaaatgtagcctccagcgggaacagctccctggctgccgagctccagcgggaggggagtcgagcgttttctttgccacttacctagtcccctgtctacaaagctggtgatcgtattagccgacttggaagactggaaaaagctggcattgatgcccagcttctcagcgatggagtaagtcctgtagattgacagcatgtactcgtggggcaccacgcgcggacccctgcctggcggctcctgcgcccggggctgctgagcccggggttcgtcctgaggccgcggctgtggttcctggccctcccggcccgcgtcactgtcgcgcggcgcccgctgcatcttgccttccttgcggcttcgcatgcccttggtggaacccagctcggcggacgacgaggaggatgagatggaagcctgctggaaaccgggcaaatcccacagaaaactgatgaggaagacggccgagagcaggaccctgggagtatccatggcgggcaagtggctgcgtctccccaggaggcggtggcggcggcgcaggacgcgcggggcacggagcggctggacagcggccggggcccggctcctcgggcggactcggagtgcgaggagccgggtcccagccacacaaaccccggccccgccacgccccctcccgcccctcgccgggaggggaggaatggggagggagggcagaggaggggtggggagggtgggaggagagccgggtggtgcgggccggaggtgtgggggagaggggccgcggtgcgccggtgtggcaggaagacgcagcgcccccgcgggacgcgcgcggggttgccgggcggtgcgcgcggcgcgggccgcaagcgctgaccgggggaaggcgggcgctgccggcccgtggccggggagcaaaggctggcccgccgcgccagggtccccctcgaactcccggaggtgtggtccctccgcagcgcggccccggctctcggtcctcgccagccgcctccactttcctgggagcgagcggccccggaggagggaagcggcggcggcgcccccaagagacagcttggagcaggcgcctctgctgcaggctgcgtgctgcctcggggcggtggtaccctccctcctcggccccaaccgccaggc

SEQ ID NO: 6 - DNA, 3089 bp, Homo sapiens
  source 1..3089: mol_type = genomic DNA
  misc_feature 1501..1589: note = chr17:48633954-48634042
ccaactcctccagctaagcaaggagcagtaactgccgtgaatcgggtggtttaatgttgttgtgttcagaaacccaggcccaacaacatgaaactacctaattcactcagcagttccaattcaagctctaggtcaagagctcactgggggcaaaccctgtggccatttttttgtgggccaaaaagcggcttaacttcattttgctccacctcttccccaacagaagaacccagttgctactaaacaacacatcggaagaactgaacccaggactctaggtaaaaccattttggagccggtcctgatagctcagattccagagacatttgctgccttccaggagccctggccagagaagaagaccctagacacaggcacaagcctgggcagggcctctttgatatacctgctcagtctctgcctctcagcccagctggaggtctccacagataaaaagaattctcaacttcaaacagatacgaaggtgcatctatactcagcaccctgctagcccctgtattccaggtcacccagcctcccagtgtagctctgagaggccagatcttcaagtcctacacaccccccagctttgagattggggctcagacaggagagtgagacaaaagagtgctgagaaagaaagtgacagagagaaaggtggaaaagcagagtgtcagaaagtttcgggaattctagggaacaaacagaggaagaatgggatttggaggggaaagccggttgatctgaacagttgctgtgaaggcaccctgcccaaaatgtcccagggccctggctctgcagaggccgagctgccccaggtaagacaattcattccgaatcttcgcagaataaggactgagaggctaaggactgggattgggacacagagaacaaatttgcttcctccttcctgaccttcggtctgggtccttggccccctaacgtgcccgctcctcacctctgcctctccagacacccgcctgctcacaggtgctcacgctcacacccgcacccatcgcaaaaacgcagctgtgcaggccgagggcggcggcggacttacctgggcggcggcggtgccggcagtgcgcggccgtcggaaggtgcggagccagcggccgcggcccagtccaggctccctcccgccctcgcccagaagcgagggtccgagtggccacgtgtccggcagggaagtccgaggtagcgagggagtccacctggccgcccgctccccctcccgggtataaatcttggggaccggaaatacaataaaacttcaccgtgttgatgaacttcaaacggtttacatcccctcctgtcctgaaaagaaagacgtccgggggcggattaaaaggaaggggaaacaaatttacgagcggcagaagcacccgcctcggcccctttctttgcccgcacactttgtccgcgtggagagaagcagccccagcccccgggacttggcctccgccgaaccggccgccaggcgcgctcttctctcggaggagtcggcgctgacccagcccgcgcccggcagagactggaagccgccgcctacacggaaaatccacagagccccgcgcagaccctatgatcggctcggcccgccgggcttgggatgaggctccctgcttctcgctagagcagaactgggctccctggcgcttccttgcgaaagcccaggctctcccaaccacgcccggtggcctccattttttgcatctttccgctgaaagcgggttttttcttttttctttttttttgacagagtcctgctgtgtcacccaggctggagtgcagtggcgcgatctcggctcactgcaacctccgcctcccggttcaagcgattctcctgcctcagcctcccgagtagctggaactacaggcgcccgccaccacgcccggctaatttttgtatttttagtagagacggggtttcacaatattggccaagctgatcttgaactcctgacctcgtgatccaccctcctcggcctcccaaagtgctgggattacaggcgtaagccaccgcgcccgacccaagggttttttgtttttgttttttgtttaactttacttttctctttccttttccgtttctagcggccagacctttgcccagccctgcccgtttattgccgggtacttgctggaaggggacagaagataagactcggggtgactcccaaggcctgaagggggctgattgggccgggggctcccagaggataaacctaggggccggtcggtcttcctcggcgtggaagtgagagccacgcggcgtggcggagctccaccaccgtctccttatctctttaaagcctcaaaatcaaacaaaaccactactacccaggcctcaagtttccacagtttttgtctgctctggaccgtttactttttttgaaaaaagagaacttggtggaatccaaattctctactaggcctccgaaccaaaacgaaggaaaatccgttttcttcttgggcttcagagaactgggatcgaagtgattgacttcctgctccttttgtctgctccaggggcctggttaggtgcccttctggatgggagagcaaaaggttctccatcctgcctcacagttattcacctccaaaacagttttgagacacaatggatggctaagattagctcaggctcaggcagagtgttcaggtacaggagtgaggtccagctgcaggcccaagagggggtttagtgcactgaaggcacccaccttcccatagatacacacatagataaccccactccccaaccccaagaaaaggcaccaaagtgctgctggatattttaaaaatctgattaaaaaataaacgggcagggaaaatactaggcagtataggttttgaattttctgaagggttaactctgctgcaggcagtcccactcggccccagctctccagaggtgggtggtggtctgggggcagtgccctctggccccttcctagcaccaaaagggaggaattggggagctctttaacagctggagggcaggaagtatcttatttctggccaacattcatattccagtatttgcatggggaggcccctccagcctccctcatttgctctttatc

SEQ ID NO: 7 - DNA, 116 bp, Homo sapiens
  source 1..116: mol_type = genomic DNA
agctggctaaagggcccttgtcccctctcagactccttcagcgggctggagtcctccctcgctcgatttcgcccgagagcgttaggggtttctaaatgcaggcgcctttgtgttgt

SEQ ID NO: 8 - DNA, 77 bp, Homo sapiens
  source 1..77: mol_type = genomic DNA
ggcgccaggaccagggggctgcccgacgccgctcgcggactagttcctcagactgtgggactccctagtgccggctt

SEQ ID NO: 9 - DNA, 89 bp, Homo sapiens
  source 1..89: mol_type = genomic DNA
agtcggcgctgacccagcccgcgcccggcagagactggaagccgccgcctacacggaaaatccacagagccccgcgcagaccctatgat

SEQ ID NO: 10 - DNA, 116 bp, synthetic construct
  source 1..116: mol_type = other DNA
agttggttaaagggtttttgtttttttttagatttttttagcgggttggagttttttttcgttcgatttcgttcgagagcgttaggggtttttaaatgtaggcgtttttgtgttgt

SEQ ID NO: 11 - DNA, 77 bp, synthetic construct
  source 1..77: mol_type = other DNA
ggcgttaggattagggggttgttcgacgtcgttcgcggattagttttttagattgtgggattttttagtgtcggttt

SEQ ID NO: 12 - DNA, 89 bp, synthetic construct
  source 1..89: mol_type = other DNA
agtcggcgttgatttagttcgcgttcggtagagattggaagtcgtcgtttatacggaaaatttatagagtttcgcgtagattttatgat

SEQ ID NO: 13 - DNA, 116 bp, synthetic construct
  source 1..116: mol_type = other DNA
agttggttaaagggtttttgtttttttttagatttttttagtgggttggagtttttttttgtttgattttgtttgagagtgttaggggtttttaaatgtaggtgtttttgtgttgt

SEQ ID NO: 14 - DNA, 77 bp, synthetic construct
  source 1..77: mol_type = other DNA
ggtgttaggattagggggttgtttgatgttgtttgtggattagttttttagattgtgggattttttagtgttggttt

SEQ ID NO: 15 - DNA, 89 bp, synthetic construct
  source 1..89: mol_type = other DNA
agttggtgttgatttagtttgtgtttggtagagattggaagttgttgtttatatggaaaatttatagagttttgtgtagattttatgat

SEQ ID NO: 16 - DNA, 116 bp, synthetic construct
  source 1..116: mol_type = other DNA
agttggttaaagggtttttgtttttttttagatttttttagygggttggagttttttttygttygatttygttygagagygttaggggtttttaaatgtaggygtttttgtgttgt

SEQ ID NO: 17 - DNA, 77 bp, synthetic construct
  source 1..77: mol_type = other DNA
ggygttaggattagggggttgttygaygtygttygyggattagttttttagattgtgggattttttagtgtyggttt

SEQ ID NO: 18 - DNA, 89 bp, synthetic construct
  source 1..89: mol_type = other DNA
agtyggygttgatttagttygygttyggtagagattggaagtygtygtttatayggaaaatttatagagtttygygtagattttatgat

SEQ ID NO: 19 - DNA, 116 bp, synthetic construct
  source 1..116: mol_type = other DNA
agytggytaaagggyyyttgtyyyytytyagaytyyttyagygggytggagtyytyyytygytygatttygyyygagagygttaggggtttytaaatgyaggygyytttgtgttgt

SEQ ID NO: 20 - DNA, 77 bp, synthetic construct
  source 1..77: mol_type = other DNA
ggygyyaggayyagggggytgyyygaygyygytygyggaytagttyytyagaytgtgggaytyyytagtgyyggytt

SEQ ID NO: 21 - DNA, 89 bp, synthetic construct
  source 1..89: mol_type = other DNA
agtyggygytgayyyagyyygygyyyggyagagaytggaagyygyygyytayayggaaaatyyayagagyyyygygyagayyytatgat

SEQ ID NO: 22 - DNA, 22 bp, synthetic construct
  source 1..22: mol_type = other DNA
agttggttaaagggtttttgtt

SEQ ID NO: 23 - DNA, 29 bp, synthetic construct
  source 1..29: mol_type = other DNA
acaacacaaaaacrcctacatttaaaaac

SEQ ID NO: 24 - DNA, 21 bp, synthetic construct
  source 1..21: mol_type = other DNA
ggygttaggattagggggttg

SEQ ID NO: 25 - DNA, 29 bp, synthetic construct
  source 1..29: mol_type = other DNA
aaaccracactaaaaaatcccacaatcta

SEQ ID NO: 26 - DNA, 18 bp, synthetic construct
  source 1..18: mol_type = other DNA
agtyggygttgatttagt

SEQ ID NO: 27 - DNA, 23 bp, synthetic construct
  source 1..23: mol_type = other DNA
atcataaaatctacrcraaactc

SEQ ID NO: 28 - DNA, 18 bp, synthetic construct
  source 1..18: mol_type = other DNA
cgttcgagagcgttaggg

SEQ ID NO: 29 - DNA, 16 bp, synthetic construct
  source 1..16: mol_type = other DNA
ttcgacgtcgttcgcg

SEQ ID NO: 30 - DNA, 19 bp, synthetic construct
  source 1..19: mol_type = other DNA
tcgcgttcggtagagattg

SEQ ID NO: 31 - DNA, 316 bp, synthetic construct
  source 1..316: mol_type = other DNA
ctgccatccctgaagccctacatccccatacacactctgtgcacatccagtgccctgctccaccatggcagtgcccgcaagggggtcccagatgagaagaagctggctaaagggcccttgtcccctctcagactccttcagcgggctggagtcctccctcgctcgatttcgcccgagagcgttaggggtttctaaatgcaggcgcctttgtgttgtaacgaaacttttagtttaagggaaaatctcttttaagccactgattgttctgacttgctgagtttactcagcagccttatgctggctctgccactgcaca

SEQ ID NO: 32 - DNA, 316 bp, synthetic construct
  source 1..316: mol_type = other DNA
ttgttatttttgaagttttatatttttatatatattttgtgtatatttagtgttttgttttattatggtagtgttcgtaagggggttttagatgagaagaagttggttaaagggtttttgtttttttttagatttttttagcgggttggagttttttttcgttcgatttcgttcgagagcgttaggggtttttaaatgtaggcgtttttgtgttgtaacgaaatttttagtttaagggaaaattttttttaagttattgattgttttgatttgttgagtttatttagtagttttatgttggttttgttattgtata

SEQ ID NO: 33 - DNA, 277 bp, synthetic construct
  source 1..277: mol_type = other DNA
cagccgggagcaccacgctggagcaaaaaagccggagggcgcagggctccagcccggctgaccatcccacccagcgcagggaccaacggaaaacccgcgcggcgccaggaccagggggctgcccgacgccgctcgcggactagttcctcagactgtgggactccctagtgccggctttgcccagggctttccaaggctgtctcatgccctagatctgccccagcagctcaggccttggactgcgaacccagtatcccgagacaccgattccatcagt

SEQ ID NO: 34 - DNA, 277 bp, synthetic construct
  source 1..277: mol_type = other DNA
tagtcgggagtattacgttggagtaaaaaagtcggagggcgtagggttttagttcggttgattattttatttagcgtagggattaacggaaaattcgcgcggcgttaggattagggggttgttcgacgtcgttcgcggattagttttttagattgtgggattttttagtgtcggttttgtttagggttttttaaggttgttttatgttttagatttgttttagtagtttaggttttggattgcgaatttagtatttcgagatatcgattttattagt

SEQ ID NO: 35 - DNA, 289 bp, synthetic construct
  source 1..289: mol_type = other DNA
tctttgcccgcacactttgtccgcgtggagagaagcagccccagcccccgggacttggcctccgccgaaccggccgccaggcgcgctcttctctcggaggagtcggcgctgacccagcccgcgcccggcagagactggaagccgccgcctacacggaaaatccacagagccccgcgcagaccctatgatcggctcggcccgccgggcttgggatgaggctccctgcttctcgctagagcagaactgggctccctggcgcttccttgcgaaagcccaggctctcccaacc

SEQ ID NO: 36 - DNA, 289 bp, synthetic construct
  source 1..289: mol_type = other DNA
tttttgttcgtatattttgttcgcgtggagagaagtagttttagttttcgggatttggttttcgtcgaatcggtcgttaggcgcgtttttttttcggaggagtcggcgttgatttagttcgcgttcggtagagattggaagtcgtcgtttatacggaaaatttatagagtttcgcgtagattttatgatcggttcggttcgtcgggtttgggatgaggttttttgtttttcgttagagtagaattgggttttttggcgtttttttgcgaaagtttaggtttttttaatt